European Patent Application EP 4 253 400 A1, published October 4, 2023. Title: Peptide Having Activity of Protecting Cell Damage From Particulate Matter and Uses Thereof. Applicant: CAREGEN CO., LTD. The sequence listing filed with the application follows.

SEQUENCE LISTING (1 sequence)

SEQ ID NO: 1 - protein, 10 aa, Artificial Sequence
  Artificial Peptide
SSNAEVLALF